European Patent Application EP 4 696 702 A1, published February 18, 2026. Title: RECOMBINANT EXPRESSION VECTOR FOR PRODUCTION OF VIRUS-LIKE PARTICLE BASED MULTIVALENT NOROVIRUS VACCINE AND FOR MANUFACTURING METHOD OF THE SAME. Applicant: InThera Inc. The sequence listing filed with the application follows.

SEQUENCE LISTING (13 sequences)

SEQ ID NO: 1 - DNA, 4341 bp, synthetic construct
  source 1..4341: mol_type = other DNA
ttctcatgtttgacagcttatcatcgataagctttaatgcggtagtttatcacagttaaattgctaacgcagtcaggcaccgtgtatgaaatctaacaatgcgctcatcgtcatcctcggcaccgtcaccctggatgctgtaggcataggcttggttatgccggtactgccgggcctcttgcgggatatcgtccattccgacagcatcgccagtcactatggcgtgctgctagcgctatatgcgttgatgcaatttctatgcgcacccgttctcggagcactgtccgaccgctttggccgccgcccagtcctgctcgcttcgctacttggagccactatcgactacgcgatcatggcgaccacacccgtcctgtggatatccggatatagttcctcctttcagcaaaaaacccctcaagacccgtttagaggccccaaggggttatgctagttattgctcagcggtggcagcagccaactcagcttcctttcgggctttgttagcagccggatccgcgacccatttgctgtccaccagtcatgctagccatatgtatatctccttcttaaagttaaacaaaattatttctagagggaaaccgttgtggtctccctatagtgagtcgtattaatttcgcgggatcgagatctcgatcctctacgccggacgcatcgtggccggcatcaccggcgccacaggtgcggttgctggcgcctatatcgccgacatcaccgatggggaagatcgggctcgccacttcgggctcatgagcgcttgtttcggcgtgggtatggtggcaggccccgtggccgggggactgttgggcgccatctccttgcatgcaccattccttgcggcggcggtgctcaacggcctcaacctactactgggctgcttcctaatgcaggagtcgcataagggagagcgtcgaccgatgcccttgagagccttcaacccagtcagctccttccggtgggcgcggggcatgactatcgtcgccgcacttatgactgtcttctttatcatgcaactcgtaggacaggtgccggcagcgctctgggtcattttcggcgaggaccgctttcgctggagcgcgacgatgatcggcctgtcgcttgcggtattcggaatcttgcacgccctcgctcaagccttcgtcactggtcccgccaccaaacgtttcggcgagaagcaggccattatcgccggcatggcggccgacgcgctgggctacgtcttgctggcgttcgcgacgcgaggctggatggccttccccattatgattcttctcgcttccggcggcatcgggatgcccgcgttgcaggccatgctgtccaggcaggtagatgacgaccatcagggacagcttcaaggatcgctcgcggctcttaccagcctaacttcgatcactggaccgctgatcgtcacggcgatttatgccgcctcggcgagcacatggaacgggttggcatggattgtaggcgccgccctataccttgtctgcctccccgcgttgcgtcgcggtgcatggagccgggccacctcgacctgaatggaagccggcggcacctcgctaacggattcaccactccaagaattggagccaatcaattcttgcggagaactgtgaatgcgcaaaccaacccttggcagaacatatccatcgcgtccgccatctccagcagccgcacgcggcgcatctcgggcagcgttgggtcctggccacgggtgcgcatgatcgtgctcctgtcgttgaggacccggctaggctggcggggttgccttactggttagcagaatgaatcaccgatacgcgagcgaacgtgaagcgactgctgctgcaaaacgtctgcgacctgagcaacaacatgaatggtcttcggtttccgtgtttcgtaaagtctggaaacgcggaagtcagcgccctgcaccattatgttccggatctgcatcgcaggatgctgctggctaccctgtggaacacctacatctgtattaacgaagcgctggcattgaccctgagtgatttttctctggtcccgccgcatccataccgccagttgtttaccctcacaacgttccagtaaccgggcatgttcatcatcagtaacccgtatcgtgagcatcctctctcgtttcatcggtatcattacccccatgaacagaaatcccccttacacggaggcatcagtgaccaaacaggaaaaaaccgcccttaacatggcccgctttatcagaagccagacattaacgcttctggagaaactcaacgagctggacgcggatgaacaggcagacatctgtgaatcgcttcacgaccacgctgatgagctttaccgcagctgcctcgcgcgtttcggtgatgacggtgaaaacctctgacacatgcagctcccggagacggtcacagcttgtctgtaagcggatgccgggagcagacaagcccgtcagggcgcgtcagcgggtgttggcgggtgtcggggcgcagccatgacccagtcacgtagcgatagcggagtgtatactggcttaactatgcggcatcagagcagattgtactgagagtgcaccatatatgcggtgtgaaataccgcacagatgcgtaaggagaaaataccgcatcaggcgctcttccgcttcctcgctcactgactcgctgcgctcggtcgttcggctgcggcgagcggtatcagctcactcaaaggcggtaatacggttatccacagaatcaggggataacgcaggaaagaacatgtgagcaaaaggccagcaaaaggccaggaaccgtaaaaaggccgcgttgctggcgtttttccataggctccgcccccctgacgagcatcacaaaaatcgacgctcaagtcagaggtggcgaaacccgacaggactataaagataccaggcgtttccccctggaagctccctcgtgcgctctcctgttccgaccctgccgcttaccggatacctgtccgcctttctcccttcgggaagcgtggcgctttctcatagctcacgctgtaggtatctcagttcggtgtaggtcgttcgctccaagctgggctgtgtgcacgaaccccccgttcagcccgaccgctgcgccttatccggtaactatcgtcttgagtccaacccggtaagacacgacttatcgccactggcagcagccactggtaacaggattagcagagcgaggtatgtaggcggtgctacagagttcttgaagtggtggcctaactacggctacactagaaggacagtatttggtatctgcgctctgctgaagccagttaccttcggaaaaagagttggtagctcttgatccggcaaacaaaccaccgctggtagcggtggtttttttgtttgcaagcagcagattacgcgcagaaaaaaaggatctcaagaagatcctttgatcttttctacggggtctgacgctcagtggaacgaaaactcacgttaagggattttggtcatgaacaataaaactgtctgcttacataaacagtaatacaaggggtgttatgagccatattcaacgggaaacgtcttgctcgaggccgcgattaaattccaacatggatgctgatttatatgggtataaatgggctcgcgataatgtcgggcaatcaggtgcgacaatctatcgattgtatgggaagcccgatgcgccagagttgtttctgaaacatggcaaaggtagcgttgccaatgatgttacagatgagatggtcagactaaactggctgacggaatttatgcctcttccgaccatcaagcattttatccgtactcctgatgatgcatggttactcaccactgcgatccccgggaaaacagcattccaggtattagaagaatatcctgattcaggtgaaaatattgttgatgcgctggcagtgttcctgcgccggttgcattcgattcctgtttgtaattgtccttttaacagcgatcgcgtatttcgtctcgctcaggcgcaatcacgaatgaataacggtttggttgatgcgagtgattttgatgacgagcgtaatggctggcctgttgaacaagtctggaaagaaatgcataagcttttgccattctcaccggattcagtcgtcactcatggtgatttctcacttgataaccttatttttgacgaggggaaattaataggttgtattgatgttggacgagtcggaatcgcagaccgataccaggatcttgccatcctatggaactgcctcggtgagttttctccttcattacagaaacggctttttcaaaaatatggtattgataatcctgatatgaataaattgcagtttcatttgatgctcgatgagtttttctaagaa

SEQ ID NO: 2 - protein, 7 aa, synthetic construct
MSAVKAA

SEQ ID NO: 3 - protein, 70 aa, synthetic construct
AAVQAAEVKVDGSEPKLSKNELKRRLKAEKKVAEKEAKQKELSEKQLSQATAAATNHTTDNGVGPEEESV

SEQ ID NO: 4 - protein, 70 aa, synthetic construct
AAVQAAEVKVDGSEPKLSANELAARLAAEAAVAEAEAAQAELSEKQLSQATAAATNHTTDNGVGPEEESV

SEQ ID NO: 5 - protein, 70 aa, synthetic construct
AAVQAAEVKVDGSEPKLSANELKRRLKAEKKVAEKEAAQAELSEKQLSQATAAATNHTTDNGVGPEEESV

SEQ ID NO: 6 - protein, 70 aa, synthetic construct
AAVQAAEVKVDGSEPKLSANELAARLKAEKKVAEKEAKQKELSEKQLSQATAAATNHTTDNGVGPEEESV

SEQ ID NO: 7 - protein, 70 aa, synthetic construct
AAVQAAEVKVDGSEPKLSKNELARRLKAEAAVAEKEAKQKELSEKQLSQATAAATNHTTDNGVGPEEESV

SEQ ID NO: 8 - protein, 70 aa, synthetic construct
AAVQAAEVKVDGSEPKLSKNELAARLKAEAAVAEKEAKQKELSEKQLSQATAAATNHTTDNGVGPEEESV

SEQ ID NO: 9 - protein, 540 aa, synthetic construct
MKMASNDAAPSNDGAAGLVPEGNNETLPLEPVAGAAIAAPVTGQNNIIDPWIRTNFVQAPNGEFTVSPRNSPGEILLNLELGPDLNPYLAHLSRMYNGYAGGVEVQVLLAGNAFTAGKILFAAVPPNFPVEFLSPAQITMLPHLIVDVRTLEPIMIPLPDVRNTFFHYSNQPNSRMRLVAMLYTPLRSNGSGDDVFTVSCRVLTRPTPDFEFTYLVPPSVESKTKPFSLPILTLSELTNSRFPVPIDSLFTAQNNVLQVQCQNGRCTLDGELQGTTQLLPSGICAFRGRVTAQINQRDRWHMQLQNLNGTTYDPTDDVPAPLGTPDFKGVVFGMVSQRNVGNDAPGSTRAQQAWVSTYSPQFVPKLGSVNLRISDNDDFQFQPTKFTPVGVNDDDDGHPFRQWELPNYSGELTLNMNLAPPVAPNFPGEQLLFFRSFVPCSGGYNQGIIDCLIPQEWIQHFYQESAPSQSDVALIRYVNPDTGRTLFEAKLHRSGYITVAHSGDYPLVVPANGHFRFDSWVNQFYSLAPMGTGNGRRRAQ

SEQ ID NO: 10 - protein, 548 aa, synthetic construct
MKMASNDAAPSNDGAAGLVPEINNEAMALEPVAGAAIAAPLTGQQNIIDPWIMNNFVQAPGGEFTVSPRNSPGEVLLNLELGPEINPYLAHLARMYNGYAGGFEVQVVLAGNAFTAGKVIFAAIPPNFPIDNLSAAQITMCPHVIVDVRQLEPINLPMPDVRNNFFHYNQGSDSRLRLIAMLYTPLRANNSGDDVFTVSCRVLTRPSPDFSFNFLVPPTVESKTKPFTLPILTISEMSNSRFPVPIDSLHTSPTENIVVQCQNGRVTLDGELMGTTQLLPSQICAFRGTLTRSTSRAGDQADTATPRLFNYYWHIQLDNLNGTPYDPAEDIPAPLGTPDFRGKVFGVASQRNPDSTTRAHEAKVDTTSGRFAPKLGSLEISTESSDFDSNQPTRFTPVGIGVDNEADFQQWSLPDYSGQFTHNMNLAPAVAPNFPGEQLLFFRSQLPSSGGRSNGILDCLVPQEWVQHFYQESAPAQTQVALVRYVNPDTGRVLFEAKLHKLGFMTIAKNGDSPITVPPNGYFRFESWVNPFYTLAPMGTGNGRRRIQ

SEQ ID NO: 11 - protein, 542 aa, synthetic construct
MKMASNDAAPSTDGAAGLVPESNNEVMALEPVAGAALAAPVTGQTNIIDPWIRANFVQAPNGEFTVSPRNAPGEVLLNLELGPELNPYLAHLARMYNGYAGGMEVQVMLAGNAFTAGKLVFAAVPPHFPVENLSPQQITMFPHVIIDVRTLEPVLLPLPDVRNNFFHYNQKDDPKMRIVAMLYTPLRSNGSGDDVFTVSCRVLTRPSPDFDFTYLVPPTVESKTKPFTLPILTLGELSNSRFPVSIDQMYTSPNEIISVQCQNGRCTLDGELQGTTQLQVSGICAFKGEVTAHLHDNDHLYNVTITNLNGSPFDPSEDIPAPLGVPDFQGRVFGIISQRDKHNSPGHNEPANRGHDAVVPTYTAQYTPKLGQIQIGTWQTDDLTVNQPVKFTPVGLNDTEHFNQWVVPRYAGALNLNTNLAPSVAPVFPGERLLFFRSYIPLKGGYGNPAIDCLLPQEWVQHFYQEAAPSMSEVALVRYINPDTGRALFEAKLHRAGFMTVSSNTSAPVVVPANGYFRFDSWVNQFYSLAPMGTGNGRRRVQ

SEQ ID NO: 12 - protein, 530 aa, synthetic construct
MMMASKDATSSVDGASGAGQLVPEVNASDPLAMDPVAGSSTAVATAGQVNPIDPWIINNFVQAPQGEFTISPNNTPGDVLFDLSLGPHLNPFLLHLSQMYNGWVGNMRVRIMLAGNAFTAGKIIVSCIPPGFGSHNLTIAQATLFPHVIADVRTLDPIEVPLEDVRNVLFHNNDRNQQTMRLVCMLYTPLRTGGGTGDSFVVAGRVMTCPSPDFNFLFLVPPTVEQKTRPFTLPNLPLSSLSNSRAPLPISSMGISPDNVQSVQFQNGRCTLDGRLVGTTPVSLSHVAKIRGTSNGTVINLTELDGTPFHPFEGPAPIGFPDLGGCDWHINMTQFGHSSQTQYDVDTTPDTFVPHLGSIQANGIGSGNYVGVLSWISPPSHPSGSQVDLWKIPNYGSSITEATHLAPSVYPPGFGEVLVFFMSKMPGPGAYNLPCLLPQEYISHLASEQAPTVGEAALLHYVDPDTGRNLGEFKAYPDGFLTCVPNGASSGPQQLPINGVFVFVSWVSRFYQLKPVGTASSARGRLGLRR

SEQ ID NO: 13 - protein, 545 aa, synthetic construct
MMMASKDAPPNMDGTSGAGQLVPEANTAEPISMEPVAGAATAAATAGQVNMIDPWIMNNYVQAPQGEFTISPNNTPGDILFDLQLGPHLNPFLSHLAQMYNGWVGNMKVKVLLAGNAFTAGKIIISCIPPGFAAQNISIAQATMFPHVIADVRVLEPIEVPLEDVRNVLFHNNDNTPTMRLVCMLYTPLRASGSSSGTDPFVIAGRVLTCPSPDFSLLFLVPPNVEQKTKPFSVPNLPLNTLSNSRVPSLIKSMMVSRDHGQMVQFQNGRVALDGQLQGTTPTSASQLCKIRGSVFHANGGNGYNPTELDGSPYHAFESPAPIGFPDLGECDWHMEASPTTQFDTGDVIKQINVKQESAFAPHLGTIQADGLSDVSVNTNMIAKLGWVSPVSDGHRGNVDPWVIPRYGSTLTEAAQLAPPIYPPGFGEAIVFFMSDFPIAHGTNGLSVPCTIPQEFVTHFVNEQAPTRGEAALLHYLDPDTHRNLGEFKLYPEGFMTCVPNSSGTGPQTLPINGVFVFVSWVSRFYQLKPVGTAGPARRLGIRRS